European Patent Specification EP 3 359 203 B1, published July 31, 2024. Title: RECEPTOR-BINDING DOMAINS LIGANDS FOR THE DETECTION, DIAGNOSIS AND TREATMENT OF PANCREATIC CANCER. Applicant: METAFORA Biosystems Centre National de la Recherche Scientifique Université de Montpellier Institut National de la Santé et de la Recherche Médicale TOUHAMI Jawida. The sequence listing filed with the application follows.

SEQUENCE LISTING (55 sequences)

SEQ ID NO: 1 - protein, 189 aa, Artificial Sequence
  HERV-W.RBD
MALPYHIFLFTVVSPSFTLTAPPPCRCMTSSSPYQEFLWRMQRPGNIDAPSYRSLCKGTPTFTAHTHMPRNCYHSATLCMHANTHYWTGKMINPSCPGGLGVTVCWTYFTQTGMSDGGGVQDQAREKHVKEVISQLTRVHGTSSPYKGLDLSKLHETLRTHTRLVSLFNTTLTGLHEVSAQNPTNCWIC

SEQ ID NO: 2 - protein, 121 aa, Artificial Sequence
  HERV-W.RBD
MALPYHIFLFTVLLPSFTLTAPPPCRCMTSSSPYQEFLWRMQRPGNIDAPSYRSLSKGTPTFTAHTHMPRNCYHSATLCMHANTHYWTGKMINPSCPGGLGVTVCWTYFTQTGMSDGGGVQ

SEQ ID NO: 3 - DNA, 363 bp, Artificial Sequence
  HERV-W.RBD
atggccctcccttatcatatttttctctttactgttcttttaccctctttcactctcactgcaccccctccatgccgctgtatgaccagtagctccccttaccaagagtttctatggagaatgcagcgtcccggaaatattgatgccccatcgtataggagtctttctaagggaacccccaccttcactgcccacacccatatgccccgcaactgctatcactctgccactctttgcatgcatgcaaatactcattattggacaggaaaaatgattaatcctagttgtcctggaggacttggagtcactgtctgttggacttacttcacccaaactggtatgtctgatgggggtggagttcaa

SEQ ID NO: 4 - protein, 316 aa, Artificial Sequence
  Xeno.RBD
MLVMEGSAFSKPLKDKINPWGPLIVMGILVRAGASVQRDSPHQIFNVTWRVTNLMTGQTANATSLLGTMTDTFPKLYFDLCDLVGDYWDDPEPDIGDGCRTPGGRRRTRLYDFYVCPGHTVPIGCGGPGEGYCGKWGCETTGQAYWKPSSSWDLISLKRGNTPKDQGPCYDSSVSSGVQGATPGGRCNPLVLEFTDAGRKASWDAPKVWGLRLYRSTGADPVTRFSLTRQVLNVGPRVPIGPNPVITDQLPPSQPVQIMLPRPPHPPPSGTVSMVPGAPPPSQQPGTGDRLLNLVEGAYQALNLTSPDKTQECWLC

SEQ ID NO: 5 - protein, 296 aa, Artificial Sequence
  Xeno.RBD
MLVMEGSAFSKPLKDKINPWGPLIVMGILVRAGASVQRDSPHQIFNVTWRVTNLMTGQTANATSLLGTMTDTFPKLYFDLCDLVGDYWDDPEPDIGDGCRTPGGRRRTRLYDFYVCPGHTVPIGCGGPGEGYCGKWGCETTGQAYWKPSSSWDLISLKRGNTPKDQGPCYDSSVSSGVQGATPGGRCNPLVLEFTDAGRKASWDAPKVWGLRLYRSTGADPVTRFSLTRQVLNVGPRVPIGPNPVITDQLPPSQPVQIMLPRPPHPPPSGTVSMVPGAPPPSQQPGTGDRLLNLVQ

SEQ ID NO: 6 - DNA, 879 bp, Artificial Sequence
  Xeno.RBD
atggaaggttcagcgttctcaaaaccccttaaagataagattaacccgtggggccccctaatagttatggggatcttggtgagggcaggagcctcggtacaacgtgacagccctcaccagatcttcaatgttacttggagagttaccaacctaatgacaggacaaacagctaacgccacctccctcctggggacgatgacagacaccttccctaaactatattttgacctgtgtgatttagtaggagactactgggatgacccagaacccgatattggggatggttgccgcactcccgggggaagaagaaggacaagactgtatgacttctatgtttgccccggtcatactgtaccaatagggtgtggagggccgggagagggctactgtggcaaatggggatgtgagaccactggacaggcatactggaagccatcatcatcatgggacctaatttcccttaagcgaggaaacactcctaaggatcagggcccctgttatgattcctcggtctccagtggcgtccagggtgccacaccggggggtcgatgcaaccccctggtcttagaattcactgacgcgggtagaaaggccagctgggatgcccccaaagtttggggactaagactctatcgatccacaggggccgacccggtgacccggttctctttgacccgccaggtcctcaatgtaggaccccgcgtccccattgggcctaatcccgtgatcactgaccagctacccccatcccaacccgtgcagatcatgctccccaggcctcctcatcctcctccttcaggcacggtctctatggtacctggggctcccccgccttctcaacaacctgggacgggagacaggctgctaaatctggtagaa

SEQ ID NO: 7 - DNA, 1059 bp, Artificial Sequence
  HERV-W.RBD fused to a mouse Fc fragment
atggccctcccttatcatatttttctctttactgttcttttaccctctttcactctcactgcaccccctccatgccgctgtatgaccagtagctccccttaccaagagtttctatggagaatgcagcgtcccggaaatattgatgccccatcgtataggagtctttctaagggaacccccaccttcactgcccacacccatatgccccgcaactgctatcactctgccactctttgcatgcatgcaaatactcattattggacaggaaaaatgattaatcctagttgtcctggaggacttggagtcactgtctgttggacttacttcacccaaactggtatgtctgatgggggtggagttcaaggatccgtcgacgtgcccagggattgtggttgtaagccttgcatatgtacagtcccagaagtatcatctgtcttcatcttccccccaaagcccaaggatgtgctcaccattactctgactcctaaggtcacgtgtgttgtggtagacatcagcaaggatgatcccgaggtccagttcagctggtttgtagatgatgtggaggtgcacacagctcagacgcaaccccgggaggagcagttcaacagcactttccgctcagtcagtgaacttcccatcatgcaccaggactggctcaatggcaaggagttcaaatgcagggtcaacagtgcagctttccctgcccccatcgagaaaaccatctccaaaaccaaaggcagaccgaaggctccacaggtgtacaccattccacctcccaaggagcagatggccaaggataaagtcagtctgacctgcatgataacagacttcttccctgaagacattactgtggagtggcagtggaatgggcagccagcggagaactacaagaacactcagcccatcatggacacagatggctcttacttcgtctacagcaagctcaatgtgcagaagagcaactgggaggcaggaaatactttcacctgctctgtgttacatgagggcctgcacaaccaccatactgagaagagcctctcccactctcctggtaaatga

SEQ ID NO: 8 - DNA, 1572 bp, Artificial Sequence
  Xeno.RBD fused to a rabbit Fc fragment
atggaaggttcagcgttctcaaaaccccttaaagataagattaacccgtggggccccctaatagttatggggatcttggtgagggcaggagcctcggtacaacgtgacagccctcaccagatcttcaatgttacttggagagttaccaacctaatgacaggacaaacagctaacgccacctccctcctggggacgatgacagacaccttccctaaactatattttgacctgtgtgatttagtaggagactactgggatgacccagaacccgatattggggatggttgccgcactcccgggggaagaagaaggacaagactgtatgacttctatgtttgccccggtcatactgtaccaatagggtgtggagggccgggagagggctactgtggcaaatggggatgtgagaccactggacaggcatactggaagccatcatcatcatgggacctaatttcccttaagcgaggaaacactcctaaggatcagggcccctgttatgattcctcggtctccagtggcgtccagggtgccacaccggggggtcgatgcaaccccctggtcttagaattcactgacgcgggtagaaaggccagctgggatgcccccaaagtttggggactaagactctatcgatccacaggggccgacccggtgacccggttctctttgacccgccaggtcctcaatgtaggaccccgcgtccccattgggcctaatcccgtgatcactgaccagctacccccatcccaacccgtgcagatcatgctccccaggcctcctcatcctcctccttcaggcacggtctctatggtacctggggctcccccgccttctcaacaacctgggacgggagacaggctgctaaatctggtagaaggatccgcaccctcgacatgcagcaagcccacgtgcccaccccctgaactcctggggggaccgtctgtcttcatcttccccccaaaacccaaggacaccctcatgatctcacgcacccccgaggtcacatgcgtggtggtggacgtgagccaggatgaccccgaggtgcagttcacatggtacataaacaacgagcaggtgcgcaccgcccggccgccgctacgggagcagcagttcgactgcacgatccgcgtggtcagcaccctccccatcgcgcaccaggactggctgaggggcaaggagttcaagtgcaaagtccacaacaaggcactcccggcccccatcgagaaaaccatctccaaagccagagggcagcccctggagccgaaggtctacaccatgggccctccccgggaggagctgagcagcaggtcggtcagcctgacctgcatgatcaacggcttctacccttccgacatctcggtggagtgggagaagaacgggaaggcagaggacaactacaagaccacgccggccgtgctggacagcgacggctcctacttcctctacagcaagctctcagtgcccacgagtgagtggcagcggggcgacgtcttcacctgctccgtgatgcacgaggccttgcacaaccactacacgcagaagtccatctcccgctctccgggtaaatga

SEQ ID NO: 9 - protein, 228 aa, Artificial Sequence
  Rabbit Fc fragment
APSTCSKPTCPPPELLGGPSVFIFPPKPKDTLMISRTPEVTCVVVDVSQDDPEVQFTWYINNEQVRTARPPLREQQFDCTIRVVSTLPIAHQDWLRGKEFKCKVHNKALPAPIEKTISKARGQPLEPKVYTMGPPREELSSRSVSLTCMINGFYPSDISVEWEKNGKAEDNYKTTPAVLDSDGSYFLYSKLSVPTSEWQRGDVFTCSVMHEALHNHYTQKSISRSPGK

SEQ ID NO: 10 - DNA, 687 bp, Artificial Sequence
  Rabbit Fc fragment
gcaccctcgacatgcagcaagcccacgtgcccaccccctgaactcctggggggaccgtctgtcttcatcttccccccaaaacccaaggacaccctcatgatctcacgcacccccgaggtcacatgcgtggtggtggacgtgagccaggatgaccccgaggtgcagttcacatggtacataaacaacgagcaggtgcgcaccgcccggccgccgctacgggagcagcagttcaacagcacgatccgcgtggtcagcaccctccccatcacgcaccaggactggctgaggggcaaggagttcaagtgcaaagtccacaacaaggcactcccggcccccatcgagaaaaccatctccaaagccagagggcagcccctggagccgaaggtctacaccatgggccctccccgggaggagctgagcagcaggtcggtcagcctgacctgcatgatcaacggcttctacccttccgacatctcggtggagtgggagaagaacgggaaggcagaggacaactacaagaccacgccggccgtgctggacagcgacggctcctacttcctctacaacaagctctcagtgcccacgagtgagtggcagcggggcgacgtcttcacctgctccgtgatgcacgaggccttgcacaaccactacacgcagaagtccatctcccgctctccgggtaaatga

SEQ ID NO: 11 - protein, 229 aa, Artificial Sequence
  Mouse Fc fragment
VDVPRDCGCKPCICTVPEVSSVFIFPPKPKDVLTITLTPKVTCVVVDISKDDPEVQFSWFVDDVEVHTAQTQPREEQFNSTFRSVSELPIMHQDWLNGKEFKCRVNSAAFPAPIEKTISKTKGRPKAPQVYTIPPPKEQMAKDKVSLTCMITDFFPEDITVEWQWNGQPAENYKNTQPIMDTDGSYFVYSKLNVQKSNWEAGNTFTCSVLHEGLHNHHTEKSLSHSPGK

SEQ ID NO: 12 - DNA, 690 bp, Artificial Sequence
  Mouse Fc fragment
gtcgacgtgcccagggattgtggttgtaagccttgcatatgtacagtcccagaagtatcatctgtcttcatcttccccccaaagcccaaggatgtgctcaccattactctgactcctaaggtcacgtgtgttgtggtagacatcagcaaggatgatcccgaggtccagttcagctggtttgtagatgatgtggaggtgcacacagctcagacgcaaccccgggaggagcagttcaacagcactttccgctcagtcagtgaacttcccatcatgcaccaggactggctcaatggcaaggagttcaaatgcagggtcaacagtgcagctttccctgcccccatcgagaaaaccatctccaaaaccaaaggcagaccgaaggctccacaggtgtacaccattccacctcccaaggagcagatggccaaggataaagtcagtctgacctgcatgataacagacttcttccctgaagacattactgtggagtggcagtggaatgggcagccagcggagaactacaagaacactcagcccatcatggacacagatggctcttacttcgtctacagcaagctcaatgtgcagaagagcaactgggaggcaggaaatactttcacctgctctgtgttacatgagggcctgcacaaccaccatactgagaagagcctctcccactctcctggtaaatga

SEQ ID NO: 13 - protein, 20 aa, Artificial Sequence
  Human IL-2 peptide signal
MYRMQLLSCIALSLALVTNS

SEQ ID NO: 14 - protein, 18 aa, Artificial Sequence
  Human albumin peptide signal
MKWVTFISLLFLFSSAYS

SEQ ID NO: 15 - protein, 18 aa, Artificial Sequence
  Human chymotrypsinogen peptide signal
MAFLWLLSCWALLGTTFG

SEQ ID NO: 16 - protein, 15 aa, Artificial Sequence
  Human trypsinogen-2 peptide signal
MNLLLILTFVAAAVA

SEQ ID NO: 17 - protein, 17 aa, Artificial Sequence
  Gaussia luciferase peptide signal
MGVKVLFALICIAVAEA

SEQ ID NO: 18 - protein, 21 aa, Artificial Sequence
  Mouse IgM peptide signal
MKFSWVMFFLMAVVTGVNSEF

SEQ ID NO: 19 - protein, 532 aa, Homo sapiens
  ASCT1
MEKSNETNGYLDSAQAGPAAGPGAPGTAAGRARRCAGFLRRQALVLLTVSGVLAGAGLGAALRGLSLSRTQVTYLAFPGEMLLRMLRMIILPLVVCSLVSGAASLDASCLGRLGGIAVAYFGLTTLSASALAVALAFIIKPGSGAQTLQSSDLGLEDSGPPPVPKETVDSFLDLARNLFPSNLVVAAFRTYATDYKVVTQNSSSGNVTHEKIPIGTEIEGMNILGLVLFALVLGVALKKLGSEGEDLIRFFNSLNEATMVLVSWIMWYVPVGIMFLVGSKIVEMKDIIVLVTSLGKYIFASILGHVIHGGIVLPLIYFVFTRKNPFRFLLGLLAPFATAFATCSSSATLPSMMKCIEENNGVDKRISRFILPIGATVNMDGAAIFQCVAAVFIAQLNNVELNAGQIFTILVTATASSVGAAGVPAGGVLTIAIILEAIGLPTHDLPLILAVDWIVDRTTTVVNVEGDALGAGILHHLNQKATKKGEQELAEVKVEAIPNCKSEEETSPLVTHQNPAGPVASAPELESKESVL

SEQ ID NO: 20 - DNA, 2102 bp, Homo sapiens
  ASCT1
cccgcactctgcgcctctcctcgcctttctcgcacctgctcctgcgccaggcccggagacccccggggcggcttcccagaacctgcggagcacaactggccgaccgacccattcattgggaacccgtcttttgccagagcccacgtcccctgccacctctagctcggagcggcgtgtagcgccatggagaagagcaacgagaccaacggctaccttgacagcgctcaggcggggcctgcggccgggcccggagctccggggaccgcggcgggacgcgcacggcgttgcgcgcgcttcctgcggcgccaagcgctggtgctgctcaccgtgtccggggtgctggcgggcgcgggcctgggcgcggcgttgcgcgggctcagcctgagccgcacgcaggtcacctacctggccttccccggcgagatgctgctccgcatgctgcgcatgatcatcctgccgctggtggtctgcagcctggtgtcgggcgccgcctcgctcgatgccagctgcctcgggcgtctgggcggcatccgtgtcgcctactttggcctcaccacactgagtgcctcggcgctcgccgtggccttggcgttcatcatcaagccaggatccggtgcgcagacccttcagtccagcgacctggggctggaggactcggggcctcctcctgtccccaaagagacggtggactctttcctcgacctggccagaaacctgtttccctccaatcttgtggttgcagctttccgtacgtatgcaaccgattataaagtcgtgacccagaacagcagctctggaaatgtaacccatgaaaagatccccataggcactgagatagaagggatgaacattttaggattggtcctgtttgctctggtgttaggagtggccttaaagaaactaggctccgaaggagaagacctcatccgtttcttcaattccctcaacgaggcgacgatggtgctggtgtcctggattatgtggtacgtacctgtgggcatcatgttccttgttggaagcaagatcgtggaaatgaaagacatcatcgtgctggtgaccagcctggggaaatacatcttcgcatctatattgggccatgttattcatggaggaattgttctgccacttatttattttgttttcacacgaaaaaacccattcagattcctcctgggcctcctcgccccatttgcgacagcatttgctacctgctccagctcagcgacccttccctctatgatgaagtgcattgaagagaacaatggtgtggacaagaggatcagcaggtttattctccccatcggggccaccgtgaacatggacggagcagccatcttccagtgtgtggccgcggtgttcattgcgcaactcaacaacatagagctcaacgcaggacagattttcaccattctagtgactgccacagcgtccagtgttggagcagcaggcgtgccagctggaggggtcctcaccattgccattatcctggaggccattgggctgcctactcatgacctgcctctgatcctggctgtggactggattgtggaccggaccaccacggtggtgaatgtggaaggggatgccctgggtgcaggcattctccaccacctgaatcagaaggcaacaaagaaaggcgagcaggaacttgctgaggtgaaagtggaagccatccccaactgcaagtctgaggaggagacatcgcccctggtgacacaccagaaccccgctggccccgtggccagtgccccagaactggaatccaaggagtcggttctgtgatggggctgggctttgggcttgcctgccagcagtgatgtcccaccctgttcacccagccgccagtcatggacacagggcactgccttgccaacttttaccctcccaagcaatgctttggcccagtcgctggcctgaggcttacctctcggcactggcattgggctccccagccggaactggttaccaaggacaaggacactctgacattcggcttgatccatgtccaggtgcaactgtgtgtacaccagggatctgtttggaaacaaccccttgagctgccaggctcaagaaatcatggactcacagggtcctgtgtggtt

SEQ ID NO: 21 - protein, 631 aa, Homo sapiens
  XPR1
MKFAEHLSAHITPEWRKQYIQYEAFKDMLYSAQDQAPSVEVTDEDTVKRYFAKFEEKFFQTCEKELAKINTFYSEKLAEAQRRFATLQNELQSSLDAQKESTGVTTLRQRRKPVFHLSHEERVQHRNIKDLKLAFSEFYLSLILLQNYQNLNFTGFRKILKKHDKILETSRGADWRVAHVEVAPFYTCKKINQLISETEAVVTNELEDGDRQKAMKRLRVPPLGAAQPAPAWTTFRVGLFCGIFIVLNITLVLAAVFKLETDRSIWPLIRIYRGGFLLIEFLFLLGINTYGWRQAGVNHVLIFELNPRSNLSHQHLFEIAGFLGILWCLSLLACFFAPISVIPTYVYPLALYGFMVFFLINPTKTFYYKSRFWLLKLLFRVFTAPFHKVGFADFWLADQLNSLSVILMDLEYMICFYSLELKWDESKGLLPNNSEERGHSDTMVFFYLWIVFYIISSCYTLIWDLKMDWGLFDKNAGENTFLREEIVYPQKAYYYCAIIEDVILRFAWTIQISITSTTLLPHSGDIIATVFAPLEVFRRFVWNFFRLENEHLNNCGEFRAVRDISVAPLNADDQTLLEQMMDQDDGVRNRQKNRSWKYNQSISLRRPRLASQSKARDTKVLIEDTDDEANT

SEQ ID NO: 22 - DNA, 4154 bp, Homo sapiens
  XPR1
ggaggaagatggcgggcgggctgctctgaagagacctcggcggcggcggaggaggagagaagcgcagcgccgcgccgcgccggggcccatgtggggaggagtcggagtcgctgttgccgccgccgcctgtagctgctggacccgagtgggagtgagggggaaacggcaggatgaagttcgccgagcacctctccgcgcacatcactcccgagtggaggaagcaatacatccagtatgaggctttcaaggatatgctgtattcagctcaggaccaggcaccttctgtggaagttacagatgaggacacagtaaagaggtattttgccaagtttgaagagaagtttttccaaacctgtgaaaaagaacttgccaaaatcaacacattttattcagagaagctcgcagaggctcagcgcaggtttgctacacttcagaatgagcttcagtcatcactggatgcacagaaagaaagcactggtgttactacgctgcgacaacgcagaaagccagtcttccacttgtcccatgaggaacgtgtccaacatagaaatattaaagaccttaaactggccttcagtgagttctacctcagtctaatcctgctgcagaactatcagaatctgaattttacagggtttcgaaaaatcctgaaaaagcatgacaagatcctggaaacatctcgtggagcagattggcgagtggctcacgtagaggtggccccattttatacatgcaagaaaatcaaccagcttatctctgaaactgaggctgtagtgaccaatgaacttgaagatggtgacagacaaaaggctatgaagcgtttacgtgtcccccctttgggagctgctcagcctgcaccagcatggactacttttagagttggcctattttgtggaatattcattgtactgaatattacccttgtgcttgccgctgtatttaaacttgaaacagatagaagtatatggcccttgataagaatctatcggggtggctttcttctgattgaattcctttttctactgggcatcaacacgtatggttggagacaggctggagtaaaccatgtactcatctttgaacttaatccgagaagcaatttgtctcatcaacatctctttgagattgctggattcctcgggatattgtggtgcctgagccttctggcatgcttctttgctccaattagtgtcatccccacatatgtgtatccacttgccctttatggatttatggttttcttccttatcaaccccaccaaaactttctactataaatcccggttttggctgcttaaactgctgtttcgagtatttacagcccccttccataaggtaggctttgctgatttctggctggcggatcagctgaacagcctgtcagtgatactgatggacctggaatatatgatctgcttctacagtttggagctcaaatgggatgaaagtaagggcctgttgccaaataattcagaagaacgaggtcactcggacactatggtgttcttttacctgtggattgtcttttatatcatcagttcctgctataccctcatctgggatctcaagatggactggggtctcttcgataagaatgctggagagaacactttcctccgggaagagattgtatacccccaaaaagcctactactactgtgccataatagaggatgtgattctgcgctttgcttggactatccaaatctcgattacctctacaactttgttgcctcattctggggacatcattgctactgtctttgccccacttgaggttttccggcgatttgtgtggaacttcttccgcctggagaatgaacatctgaataactgtggtgaattccgtgctgtgcgggacatctctgtggcccccctgaacgcagatgatcagactctcctagaacagatgatggaccaggatgatggggtacgaaaccgccagaagaatcggtcatggaagtacaaccagagcatatccctgcgccggcctcgcctcgcttctcaatccaaggctcgtgacactaaggtattgatagaagacacagatgatgaagctaacacttgaattttctgaagtctagcttaacatctttggttttcctactctacaatcctttcctcgaccaacgcaacctctagtacctttccagccgaaaacaggagaaaacacataacacattttccgagctcttccggatcggatcctatggactccaaacaagctcactgtgtttcttttcttttcttctggtttaattttaattttctattttcaaaacaaatatttacttcatttgccaatcagaggatgttttaagaaacaaaacatagtatcttatggattgtttacaatcacaaggacatagatacctatcaggatgaagaacaggcattgcaaggaccctctgatgggacggtactgagatatctcggcttccgctcagcccggttttgactggttgaaaccggacattggtttttaaattttttgtcagtttatgtggagaatttttttctttccttcatacccagcgcaaaggcactggccgcacttgcaggaaaagtgcaacttaaagcagtaccttcattcatgaagctactttttaatttgatgtaacttttcttattttgggaagggttgctgggtgggtgggaaatatgatgtatttgttacacatagttttctcattatttatgaaacttaaccatacagaatgatataactcctgtgcaatgaaggtgataacagtaaaagaaggcaggggaaacttacgttggatgacatttatgagggtcagtcccacatacctctttcaggagacaacttgcaccagtttgaccttttcttttctttgtttttattttaagccaaagtttcattgctaacttcttaagttgctgctgctttagagtcctgagcatatctctcgtaacaaggaatcccacacttcacaccaccggctgaatttcatggaagaggttctgataatttttttaactttttaaggaacagatgtggaatacactggcccatatttcaaccttaacagctgaagctatgccttattatgcatccacatgtatggtccctgtagcgtgacctttactagctctgaatcagaagacagagctatttcagaggctctgtgtgccctcactagatagtttttcttctgggttcaaccactttagccagaatttgatcaaattaaaagtctgtcatggggaaactatatttttgagcacatggaacaaattatacttcctcattcatattatgttgatacaaaagaccttggcagccatttctcccagcagttttaaaggatgaacattggatttcatgccatcccatagaaaacctgttttaaaattttagggatctttacttggtcatacatgaaaagtacactgcttagaaattatagactattatgatctgtccacagtgcccattgtcacttctttgtctcatttcttccctttgttccttagtcatccaaataagcctgaaaaccataagagatattactttattgaatatggttggcattaaatttagcatttcattatctaacaaaattaatataaattccaggacatggtaaaatgtgttttaataacccccagacccaaatgaaaatttcaaagtcaataccagcagattcatgaaagtaaatttagtcctataattttcagcttaattataaacaaaggaacaaataagtggaagggcagctattaccattcgcttagtcaaaacattcggttactgccctttaatacactcctatcatcagcacttccaccatgtattacaagtcttgacccatccctgtcgtaactccagtaaaagttactgttactagaaaatttttatcaattaactgacaaatagtttctttttaaagtagtttcttccatctttattctgactagcttccaaaatgtgttccctttttgaatcgaggtttttttgttttgttttgttttctgaaaaaatcatacaactttgtgcttctattgcttttttgtgttttgttaagcatgtcccttggcccaaatggaagaggaaatgtttaattaatgctttttagtttaaataaattgaatcatttataataaaaaaaaaaaaaaaaaaaaaaaaaaaaaa

SEQ ID NO: 23 - DNA, 20 bp, Artificial Sequence
  XPR1 PCR forward primer
agagcttgggagacaaagca

SEQ ID NO: 24 - DNA, 20 bp, Artificial Sequence
  XPR1 PCR reverse primer
gtggacacaacattcgcaac

SEQ ID NO: 25 - DNA, 17 bp, Artificial Sequence
  ASCT2 PCR forward primer
atcgtggagatggagga

SEQ ID NO: 26 - DNA, 18 bp, Artificial Sequence
  ASCT2 PCR reverse primer
aagaggtcccaaaggcag

SEQ ID NO: 27 - DNA, 693 bp, Artificial Sequence
  Human IgG2 Fc fragment
atatcggccatggttagatctgtggagtgcccaccgtgcccagcaccacctgtggcaggaccgtcagtcttcctcttccccccaaaacccaaggacaccctcatgatctcccggacccctgaggtcacgtgcgtggtggtggacgtgagccacgaagaccccgaggtccagttcaactggtacgtggacggcgtggaggtgcataatgccaagacaaagccacgggaggagcagttcaacagcacgttccgtgtggtcagcgtcctcaccgttgtgcaccaggactggctgaacggcaaggagtacaagtgcaaggtctccaacaaaggcctcccagcccccatcgagaaaaccatctccaaaaccaaagggcagccccgagaaccacaggtgtacaccctgcccccatcccgggaggagatgaccaagaaccaggtcagcctgacctgcctggtcaaaggcttctaccccagcgacatcgccgtggagtgggagagcaatgggcagccggagaacaactacaagaccacacctcccatgctggactccgacggctccttcttcctctacagcaagctcaccgtggacaagagcaggtggcagcaggggaacgtcttctcatgctccgtgatgcatgaggctctgcacaaccactacacgcagaagagcctctccctgtctccgggtaaatga

SEQ ID NO: 28 - protein, 239 aa, Artificial Sequence
  RD114.RBD
MKLPTGMVILCSLIIVRAGFDDPRKAIALVQKQHGKPCECSGGQVSEAPPNSIQQVTCPGKTAYLMTNQKWKCRVTPKISPSGGELQNCPCNTFQDSMHSSCYTEYRQCRRINKTYYTATLLKIRSGSLNEVQILQNPNQLLQSPCRGSINQPVCWSATAPIHISDGGGPLDTKRVWTVQKRLEQIHKAMTPELQYHPLALPKVRDDLSLDARTFDILNTTFRLLQMSNFSLAQDCWLC

SEQ ID NO: 29 - protein, 222 aa, Artificial Sequence
  RD114.RBD
MKLPTGMVILCSLIIVRAGFDDPRKAIALVQKQHGKPCECSGGQVSEAPPNSIQQVTCPGKTAYLMTNQKWKCRVTPKISPSGGELQNCPCNTFQDSMHSSCYTEYRQCRRINKTYYTATLLKIRSGSLNEVQILQNPNQLLQSPCRGSINQPVCWSATAPIHISDGGGPLDTKRVWTVQKRLEQIHKAMTPELQYHPLALPKVRDDLSLDARTFDILNTTF

SEQ ID NO: 30 - DNA, 669 bp, Artificial Sequence
  RD114.RBD
atgaaactcccagcaggaatggtcattttatgtagcctaataatagttcgggcagggtttgacgacccccgcaaggctatcgcattagtacaaaaacaacatggtaaaccatgcgaatgcagcggagggcaggtatccgaggccccaccgaactccatccaacaggtaacttgcccaggcaagacggcctacttaatgaccaaccaaaaatggaaatgcagagtcactccaaaaaatctcacccctagcgggggagaactccagaactgcccctgtaacactttccaggactcgatgcacagttcttgttatactgaataccggcaatgcagggcgaataataagacatactacacggccaccttgcttaaaatacggtctgggagcctcaacgaggtacagatattacaaaaccccaatcagctcctacagtccccttgtaggggctctataaatcagcccgtttgctggagtgccacagcccccatccatatctccgatggtggaggacccctcgatactaagagagtgtggacagtccaaaaaaggctagaacaaattcataaggctatgcatcctgaacttcaataccaccccttagccctgcccaaagtcagagatgaccttagccttgatgcacggacttttgatatcctgaataccactttt

SEQ ID NO: 31 - DNA, 1365 bp, Artificial Sequence
  RD114.RBD fused to a mouse Fc fragment
atgaaactcccagcaggaatggtcattttatgtagcctaataatagttcgggcagggtttgacgacccccgcaaggctatcgcattagtacaaaaacaacatggtaaaccatgcgaatgcagcggagggcaggtatccgaggccccaccgaactccatccaacaggtaacttgcccaggcaagacggcctacttaatgaccaaccaaaaatggaaatgcagagtcactccaaaaaatctcacccctagcgggggagaactccagaactgcccctgtaacactttccaggactcgatgcacagttcttgttatactgaataccggcaatgcagggcgaataataagacatactacacggccaccttgcttaaaatacggtctgggagcctcaacgaggtacagatattacaaaaccccaatcagctcctacagtccccttgtaggggctctataaatcagcccgtttgctggagtgccacagcccccatccatatctccgatggtggaggacccctcgatactaagagagtgtggacagtccaaaaaaggctagaacaaattcataaggctatgcatcctgaacttcaataccaccccttagccctgcccaaagtcagagatgaccttagccttgatgcacggacttttgatatcctgaataccacttttggatccgtcgacgtgcccagggattgtggttgtaagccttgcatatgtacagtcccagaagtatcatctgtcttcatcttccccccaaagcccaaggatgtgctcaccattactctgactcctaaggtcacgtgtgttgtggtagacatcagcaaggatgatcccgaggtccagttcagctggtttgtagatgatgtggaggtgcacacagctcagacgcaaccccgggaggagcagttcaacagcactttccgctcagtcagtgaacttcccatcatgcaccaggactggctcaatggcaaggagttcaaatgcagggtcaacagtgcagctttccctgcccccatcgagaaaaccatctccaaaaccaaaggcagaccgaaggctccacaggtgtacaccattccacctcccaaggagcagatggccaaggataaagtcagtctgacctgcatgataacagacttcttccctgaagacattactgtggagtggcagtggaatgggcagccagcggagaactacaagaacactcagcccatcatggacacagatggctcttacttcgtctacagcaagctcaatgtgcagaagagcaactgggaggcaggaaatactttcacctgctctgtgttacatgagggcctgcacaaccaccatactgagaagagcctctcccactctcctggtaaatga

SEQ ID NO: 32 - protein, 224 aa, Artificial Sequence
  H2.RBD
MGNVFFLLLFSLTHFPLAQQSRCTLTVGISSYHSSPCSPTQPVCTWNLDLNSLTTDQRLHPPCPNLITYSGFHKTYSLYLFPHWIKKPNRQGLGYYSPSYNDPCSLQCPYLGCQSWTCPYTGPVSSPSWKFHSDVNFTQEVSQVSLRLHFSKCGSSMTLLVDAPGYDPLWFITSEPTQPPPTSPPLVHDSDLEHVLTPSTSWTTKILKFIQLTLQSTNYSCMVC

SEQ ID NO: 33 - protein, 541 aa, Homo sapiens
  ASCT2
MVADPPRDSKGLAAAEPTANGGLALASIEDQGAAAGGYCGSRDQVRRCLRANLLVLLTVVAVVAGVALGLGVSGAGGALALGPERLSAFVFPGELLLRLLRMIILPLVVCSLIGGAASLDPGALGRLGAWALLFFLVTTLLASALGVGLALALQPGAASAAINASVGAAGSAENAPSKEVLDSFLDLARNIFPSNLVSAAFRSYSTTYEERNITGTRVKVPVGQEVEGMNILGLVVFAIVFGVALRKLGPEGELLIRFFNSFNEATMVLVSWIMWYAPVGIMFLVAGKIVEMEDVGLLFARLGKYILCCLLGHAIHGLLVLPLIYFLFTRKNPYRFLWGIVTPLATAFGTSSSSATLPLMMKCVEENNGVAKHISRFILPIGATVNMDGAALFQCVAAVFIAQLSQQSLDFVKIITILVTATASSVGAAGIPAGGVLTLAIILEAVNLPVDHISLILAVDWLVDRSCTVLNVEGDALGAGLLQNYVDRTESRSTEPELIQVKSELPLDPLPVPTEEGNPLLKHYRGPAGDATVASEKESVM

SEQ ID NO: 34 - DNA, 1626 bp, Homo sapiens
  ASCT2
atggtggccgatcctcctcgagactccaaggggctcgcagcggcggagcccaccgccaacgggggcctggcgctggcctccatcgaggaccaaggcgcggcagcaggcggctactgcggttcccgggaccaggtgcgccgctgccttcgagccaacctgcttgtgctgctgacagtggtggccgtggtggccggcgtggcgctgggactgggggtgtcgggggccgggggtgcgctggcgttgggcccggagcgcttgagcgccttcgtcttcccgggcgagctgctgctgcgtctgctgcggatgatcatcttgccgctggtggtgtgcagcttgatcggcggcgccgccagcctggaccccggcgcgctcggccgtctgggcgcctgggcgctgctctttttcctggtcaccacgctgctggcgtcggcgctcggagtgggcttggcgctggctctgcagccgggcgccgcctccgccgccatcaacgcctccgtgggagccgcgggcagtgccgaaaatgcccccagcaaggaggtgctcgattcgttcctggatcttgcgagaaatatcttcccttccaacctggtgtcagcagcctttcgctcatactctaccacctatgaagagaggaatatcaccggaaccagggtgaaggtgcccgtggggcaggaggtggaggggatgaacatcctgggcttggtagtgtttgccatcgtctttggtgtggcgctgcggaagctggggcctgaaggggagctgcttatccgcttcttcaactccttcaatgaggccaccatggttctggtctcctggatcatgtggtatgcccctgtgggcatcatgttcctggtggctggcaagatcgtggagatggaggatgtgggtttactctttgcccgccttggcaagtacattctgtgctgcctgctgggtcacgccatccatgggctcctggtactgcccctcatctacttcctcttcacccgcaaaaacccctaccgcttcctgtggggcatcgtgacgccgctggccactgcctttgggacctcttccagttccgccacgctgccgctgatgatgaagtgcgtggaggagaataatggcgtggccaagcacatcagccgtttcatcctgcccatcggcgccaccgtcaacatggacggtgccgcgctcttccagtgcgtggccgcagtgttcattgcacagctcagccagcagtccttggacttcgtaaagatcatcaccatcctggtcacggccacagcgtccagcgtgggggcagcgggcatccctgctggaggtgtcctcactctggccatcatcctcgaagcagtcaacctcccggtcgaccatatctccttgatcctggctgtggactggctagtcgaccggtcctgtaccgtcctcaatgtagaaggtgacgctctgggggcaggactcctccaaaattacgtggaccgtacggagtcgagaagcacagagcctgagttgatacaagtgaagagtgagctgcccctggatccgctgccagtccccactgaggaaggaaaccccctcctcaaacactatcgggggcccgcaggggatgccacggtcgcctctgagaaggaatcagtcatgtaa

SEQ ID NO: 35 - protein, 331 aa, Artificial Sequence
  RD114.RBD
MKPPAGMVFLWVLTSLGAGIGAKIVKEGNPHQVYTLTWQIYSQSGEVVWEVQGNHALNTWWPPLTPDFCQLAAGLDTWDIPARSPKNLQSYMGERIQQMTAHGCSSPTARCRLAQAEFYVCPRDNRDRATAHRCGGYEEYFCSAWGCETTGDAYWQPTSSWDLITITRGYTKPDPDGHTCYYKKGTEGYHHWISPLSLPLKITFTDSGKRALGWQTGYTWGLRWYLPGKDRGIVLKIKLKIDTITQTVGPNLVLADQKAPVQLAIPVQPPRAPTQTPGINPVNSTLSPSLGYPTPPLDRAQGDRLLNLVQGVYLTLNLTAPNQTQDCWLCL

SEQ ID NO: 36 - DNA, 2775 bp, Artificial Sequence
  RD114.RBD
cttcttaccccgcccaaccgtttcgggctcaccccgtatgaaatcctttatgggggacccccccctttgtcaaccttgctcaattccttctccccctccgatcctaagactgatttacaagcccgactaaaagggctgcaagcggtgcaggcccaaatctggacacccctggccgaactgtaccggccaggacatccacaaactagccacccatttcaggtaggagactccgtgtacgtccagcggcaccgctctcaaggattggagcctcgttggaagggaccttacatcgtcctgctgaccacgcccaccgccataaaggttgacgggatcgccgcctggattcacgcatcgcacgccaaggcagccccaagaacccctggaccgaaagctcccaaaacctggaagctccaccgttcggagaaccctcttaagataagactctcccgtgtctgactgttaatccaccctgtccctgcacaaacccaaaatgaaacccccagcgggaatggtctttctgtgggtcctcacaagcttgggggcgggaattggagctaaaattgtcaaagaggggaacccacatcaggtttataccttgacttggcaaatctactcccagagcggggaagttgtctgggaggtccaaggtaaccatgcgcttaatacttggtggcccccacttacccctgatttttgccagctggcagctggattagacacttgggatatcccagctagaagccccaagaacctgcagtcctacatgggggaaagaatccagcagatgactgcccatggatgcagtagtcccactgccagatgtagattagcccaggcagagttctatgtctgtcctcgagacaatagggatagggccactgcccaccgatgtgggggatatgaagaatatttctgctcggcatggggctgcgaaactactggcgatgcctactggcaacctacctcttcctgggacttaatcaccattacaagaggttacaccaaacctgaccccgatggacacacttgctactataaaaagggcacagaagggtatcatcattggataagtcccctgtctctacctcttaagattacctttacagattcaggaaaacgggctctcggatggcagacgggctatacatggggactccgatggtacctaccgggaaaagatagggggattgttctaaaaatcaaattaaaaatagatacaatcacccaaaccgtaggtcccaacctagtattggccgatcaaaaagctccggtccagctagccatcccagtccagccaccaagggccccaactcagacaccgggaattaaccctgttaattccactctaagccccagtctaggatacccgaccccccctctcgaccgggcacaaggagataggctcctaaaccttgtacaaggggtatacttaactctcaaccttacggccccaaatcaaactcaggactgttggctctgcctaacggctaaacccccttactatcagggagttgctataattgggaactttactaaccatacgaatgccccactgagatgtagcactacacctcgacatggcctcactttaactgaagtcaccggtcatggcctatgtattgggaaaattccaccctcacaccagaatctctgtagtcagaccataccatctgtcgggcagggtccctattatttgaccgctcccaacggaacgtactgggtctgtaacaccggactcacgccatgcatctcgctccaggtactcaataatactgccgactattgcatcctaattgaactttggccaaaaatcttctaccatgactcagaatatatttatggccactacgaacccggcggcagattccggagagaaccagtttccctcaccgtagcactgctcctagggggattaactatgggaagtttagcagctggcatagggacaggcaccgcagctctcatagaaactaatcagttcaagcagttacaaatcgctatgcattctgacatacaggcactagaagaatccatctcggcactagaaagatccctaacctccctctcagaagtggttttacaaaatcggaggggacttgacctgttgttcttacaagaaggcgggttatgtgctgccctcaaagaagagtgctgcttctatgctgatcacacaggaatagtgagagacagcatggccaagctgagggagagactcaaacaaagacaaaagctgttcgaatctcagcaaggctggtttgaggggtggtataacaaatccccctggtttaccactctagtctcctccctcatgggccctttaatactcctactattaatactgatgttcggaccttgcatcctcaaccgcttggtacaattcataagagaaagactctctgtcatccaggccttggtcctaactcaacagtaccaccaactaagacaatttgacgcagaaaggccagatacaatcgaatgaaaggtttcattcgacgccaaaagaaaatgggggaatgaaagacccctgcttagcttaataacacacccccaccctatcttcagttccgtaacgcctcacttgcagggcttgcacttccaccagttgacaaacaggatatctgcagttagacatccgtaccctgggagagctgtacccccacctttccctacgcaagacaggaacaggttgtcacataaataacgatgaccgctttcatctcgcttctgtaaacctgcttacgctcccaaaccggaggtcccctgccgcttcgcacc

SEQ ID NO: 37 - protein, 222 aa, Artificial Sequence; identical to SEQ ID NO: 29
  RD114.RBD

SEQ ID NO: 38 - protein, 181 aa, Artificial Sequence
  HERV-W.RBD
MALPYHIFLFTVLLPSFTLTAPPPCRCMTSSSPYQEFLWRMQRPGNIDAPSYRSLSKGTPTFTAHTHMPRNCYHSATLCMHANTHYWTGKMINPSCPGGLGVTVCWTYFTQTGMSDGGGVQDQAREKHVKEVISQLTRVHGTSSPYKGLDLSKLHETLRTHTRLVSLFNTTLTGLHEVSAQ

SEQ ID NO: 39 - protein, 239 aa, Artificial Sequence
  BaEV.RBD
MGFTTKIIFLYNLVLVYAGFDDPRKAIELVQKRYGRPCDCSGGQVSEPPSDRVSQVTCSGKTAYLMPDQRWKCKSIPKDTSPSGPLQECPCNSYQSSVHSSCYTSYQQCRSGNKTYYTATLLKTQTGGTSDVQVLGSTNKLIQSPCNGIKGQSICWSTTAPIHVSDGGGPLDTTRIKSVQRKLEEIHKALYPELQYHPLAIPKVRDNLMVDAQTLNILNATYNLLLMSNTSLVDDCWLC

SEQ ID NO: 40 - protein, 251 aa, Artificial Sequence
  SRV.RBD
MNFNHHFTWSLVIISQIFQVQAGFGDPREALLEIQQKHGKPCDCAGGYVSSPPTNSLTTVSCSTYTAYSVTNSLKWQCVSTPTTASPTHIGSCPSQCNSQSYDSVHATCYNHYQQCTIGNKTYLTATMIRDKSPSSGDGNVPTILGNNQNLIIAGCPENKKGQVVCWNSQPSVHMSDGGGPQDKVREIIVNKKFEELHKSLFPELSYHPLALPEARGKEKIDAHTFDLLATVHSLLNVSSQRQLAEDCWLC

SEQ ID NO: 41 - DNA, 8173 bp, Artificial Sequence
  SRV.RBD
cctgtccggagccgtgctgcccggatgatgtcttggcctctgtttgctctagctctacgcttaagattcaagatggcgaacttcctggttcttctctgtgttgctttcccgccggcgcgaatgtttcccgctcttaggcttacgtggctttcccagttctgcagttgagcatgcgcccagtacttctcccctcccacttactgcctgtgtatataagacaacgcattgccaccattaaacgagacttgatcagaacactgtcttgtctccatttcttgtgtctcttgtcccatccaattcccactccctcctccaggtttcctactgttggtcccgcgggacgggacatttggcgcccaacgtggcgttggatacgagggaatttcgtgaggaagacgacgcggtttgccggcccggattaaaagagaaacgaaagtaaactttcttcggccgccgcgggagcctgccgcgtaggacctgaaagtaagtggtgcgctcggatatggggcaggaattaagccagcacgaacgttatgtggaacaattaaaacaggctttaaagacacggggagtaaaggttaaatatgctgatctcttaaagttttttgattttgtaaaggatacttgtccttggtttccgcaagagggaaccatagatatcaaaaggtggcgtagagtaggcgattgtttccaagattattataatacttttggccctgagaaagtcccagtaactgccttctcatactggaatttaattaaagaattgatagataagaaagaagttaacccacaagtaatggctgccgtggctcaaactgaagaaatcttaaaaactagttctcatacagagcttacaacaaagccctcccaaaatccagacttggaccttatttctcttgatagtgacgatgaaggagctaaaggttcctccctaaaagataaaaatttatcatgtactaaaaagccaaaaagattcccagttctattaacagcacaaactagtgcggaccctgaggaccccaacccctcagaggtagactgggacggattagaggatgaggcagcaaaatatcataatcccgattggcctcccttcctaacccgtccacctccttataataaagccactccttccgcacccactgtaatggcggttgttaatccaaaagaggaattaaaagagaagattgctcaattagaggaacagattaaattagaagagttacatcaagcactcatttccaagttacaaaaactaaaaacaggaaatgaaactgtcactagtccagaaactgcagggggcttttctcgcacacctcactggccggggcaacatatccctaaaggaaaatgctgcgccagtcgagaaaaggaagaacaaaccccaaaagatattttcccagtaactgaaactgtcgatgggcagggtcaagcctggaggcaccataatggttttgattttaccgtcataaaagaattaaaaacggctgcctctcaatatggggctactgccccatacacattagccatagtagaatctgtagcggacaattggcttacccctacagattggaatacacttgttagggcagtcctctcaggaggagatcatttactatggaaatctgagttttttgaaaattgtagagaaacggctaaaagaaatcaacaagccggtaatggttgggattttgatatgttaacaggctcaggtaactattctagcactgatgcacaaatgcaatatgatccgggattgtttgctcaaattcaagcggctgctacaaaagcctggagaaaacttcccgttaagggagacccaggagcttcccttacaggagtcaaacaaggacccgatgagccatttgcagattttgtacacagacttataacaactgctgggagaatttttggaagtgctgaggctggtgtagactatgtaaaacaactagcatatgaaaacgctaatccagcctgtcaggcagccatccgcccctatagaaagaaaacagatttaactggctacatccgcctttgttcggacattgggccttcttatcaacagggcttagccatggccgccgcctttagcggacaaactgtcaaagattttcttaacaacaaaaataaagaaaaaggagggtgttgttttaaatgcgggaggaaaggacattttgcaaaaaattgtcatgaacatatacataacaattctgaaacaaaggctcctggactctgtcccaggtgtaaaagagggaaacattgggccaatgaatgcaaatccaaaactgatagtcaaggaaacccactaccaccccatcagggaaacggactgaggggccagccccaggccccgaaacaagcttatggggcggtcagctttgttccagccaacaaaaacaacccatttcaaagcttaccagagccaccccaggaagtgcaggattggacctcagttccacctcccacacagtattaacaccggaaatggggccccaagcgttaagcactggaatatatgggcccctacctcccaacacttttggattaatcttaggcagaagtagcattactataaaaggtctacaagtttatccaggagtaattgataatgactatactggggaaattaaaataatggcaaaggctgtcaacaatattgttactgttcctcaaggcaacaggatagctcaattaatcctcctacctctaattgagacagacaataaagtacaacaaccctatagaggacaaggaagttttggatcctcagacatatattgggtccaacctattacctgtcagaagccctccttaacattatggttagatgataaaatgttcacaggattaatcgatacgggagctgatgtcactatcatcaagctagaggactggcctcctaattggcctataacagataccttaaccaatttaagaggtataggacaaagcaacaaccctaagcaaagttctaaatatcttacttggagagataaagaaaataattctggtctcattaaaccgtttgttattcctaatttacctgtcaacctttggggcagagatctcctttctcaaatgaaaattatgatgtgtagtcctagtgacatagtcactgcccaaatgttagcccaaggctacagccccggaaaaggattaggaaaaaacgaaaatggcattctacatcctatcccaaatcaaggacaatttgacaaaaagggatttggaaatttttaactgcggccattgacatgcttgcaccccaacagtgtgctgaacccatcacgtggaaatcagacgaacctgtctgggttgatcagtggccattaaccagtgaaaaacttgctgctgcccaacagttagtgcaagaacagttagaggcaggacatattactgaaagtaattccccttggaacactcccatatttgttataaaaaagaaatctggtaaatggaggctcttacaagatttacgagccgttaatgccactatggtattaatgggagctttacaacctggattgccctctccggtggctatcccacaagggtatcttaaaataattattgatctcaaagattgtttcttttctattccccttcatcctagtgatcaaaaaaggtttgcattcagcctaccttccacaaattttaaggaacctatgcaacgttttcagtggaaagttttaccgcaacgtatggccaacagccctaccttatgccaaaaatatgtggccacagccatacataaagttagacatgcctggaaacaaatgtatattatacattacatggatgatatcctcatagctggtaaagatggacaacaagttttacaatgctttgatcagctcaaacaagaattgactatagccgggttacatatagccccagaaaaaattcaactacaagacccctacacgtatttaggatttgaacttaatggtccaaaaatcactaatcaaaaggcagttattcgtaaagataagttgcaaactcttaatgactttcaaaagcttttaggagacatcaattggctccgaccatacctgaaactcactactgcagatttaaaacctttattcgacacccttaaaggagactctaatcccaattctcatagatctttatcaaaagaagctcttgccttacttgataaagtagaaacagccattgcagaacaatttgttactcacataaattattcattaccattaatgtttctcatatttaacacagccctgacgcccactggtttattttggcagaataatcctattatgtgggtccacctgcctgcatcccctaaaaaggtattactcccctattacgacgctatagcagatttaatcatactaggaagagaccatagtaaaaaatactttggaattgaaccctccgtaatcatacagccatactctaagtctcaaattgattggctgatgcaaaacactgaaatgtggccaattgcctgtgcctcttatgttggcatcctagataaccattacccacctaacaagcttatccaattctgcaaattacatgcctttattttccctcaaatcattagtaaaacgcccttaaacaatgctttattagtttttactgatggctcttccactggaatggccgcatatactcttgctgatactaccatcaaatttcaaactaatcttaattcggctcaactagtagaattacaagccttaattgcagtcctatcagctttccccaaccaacctcttaacatttatactgacagtgcttacttagcccactcaatacccctgcttgaaactgtagcacaaattaaacacatatcagaaacagcaaagctattcctacagtgccaacagcttatatacaatagatccatacctttttacatcggacatgtcagggcccattctggcctacctggacctatagcccacggcaaccaaaaggctgacttggcaactaaaaccgtggctagcaacataaacacaaacctcgaatcggctcaaaatgctcataccttacatcatctcaatgcccaaactttaaaactaatgtttaacattccgagagaacaagctagacaaattgtcagacaatgcccaatatgtgcaacctatctaccagtccctcatttaggagttaatcctagaggattgttgcccaacatgatttggcaaatggacgttacacattactccgaatttggtaatttaaaatatatacatgtttctatagataccttcagtggattcctattagccactctacagacaggagaaacaacaaaacatgtcataacccatttacttcattgcttctctattattggactccctaaacaaataaaaacagataacggtcctggatacacctccaaaaattttcaagaattctgctccacacttcaaattaaacatgttactggaatcccctataatccccaaggccaaggaatagttgaaagagcccacttatctcttaaaaccaccattgaaaaaataaaaaagggggaatggtaccctacgaagggtacccccaggaacattctcaatcatgcactctttattctaaattttttaaatttggatgatcaaaaccactcagcagctgatcgtttttggcatagcaaccccagaaaacaatttgccatggtaaaatggaaagatccactagacaatacgtggccatggcctgatccagtgataatttggggcagaggttcagtctgtgtttactctcaaacccatgatgccgctagatggctaccagaacgactagtaaaacaaatacctaacaataaccaatccagggagtgattctctccctgagattgccttttcctttgctcacagagatgaacttcaatcatcatttcacctggagcttagtgataatatctcaaatattccaagttcaagccggttttggagatccgcgcgaggccctcctagagatacaacaaaaacatggtaagccttgtgactgtgctggaggatatgtttccagtccacctactaattcccttacaactgtctcatgctctacttatactgcttattcagtaaccaactccctaaagtggcagtgtgtgtctactcccactacagccagccccacacatataggatcttgtcccagtcaatgtaactcacaatcatatgactctgtacatgccacctgctataaccactatcaacaatgtactattggtaataagacatatctcactgctactatgattagagacaaatctccctccagtggtgacgggaacgtccctacaatattagggaataatcaaaacctcattatagcaggctgtcccgaaaataaaaagggccaagtggtttgctggaatagccaaccctctgttcacatgtctgatggaggagggcctcaagataaggtccgtgagattatagtaaataaaaagtttgaagaattgcataaatcgctgttcccagaactttcttaccaccctctggctttgcccgaagcccgtggtaaagaaaaaattgatgcacacacttttgatctccttgccactgtgcatagtttactcaatgtttcctcccaacgccaattagccgaagattgctggctgtgcttgcggtcaggtgatcccgttcctctcgccctgccttatgataacacatcctgctctaactcaacctttttctttaattgctctaattgctcttgccttatcaccccccctttcttagtacagccctttaacttcactcattctgtttgcctttacgctgattatcaaaacaactcatttgacatagatgtaggtctagctggcttcactaattgctctagttatattaatatttctaaaccctccagtcccttatgcgccccaaatagctcagtttttgtatgcggtaataacaaggcatacacttatctacccacaaattggacgggaagctgtgtacttgctactcttttacccgatatagacattattccaggtagtgaacctgtccccattccagctatagatcattttttaggtagacccaaaagagcaatccagtttattcccctagtcataggattaggtataactactgcagtatctaccgggactgctggtctgggggtttccctcactcaatacacaaaattgtctcaccaactaatatcagatgtacaagctatttctagtactatacaagatctccaagatcaagtagactctctagcagaagtagtactacaaaacagaagaggattagatctgctgacagcagagcagggaggcatctgcttagctttacaggaaaaatgctgtttctacgccaacaaatctggaatcgtcagagacaagattaaaaacctacaagatgacttagaaaaacgccgaaaacaactgatcgacaaccccttttggactggctttcatggactcctcccttatgttatgcctctattaggccctttactttgcttactgcttgtgttatctttcggaccaattatcttcaataagcttatgacttttattaaacatcaaatcgagagcattcaagccaaacctatacaggtccattatcatcgccttgaacaagaagaccatggtggctcatatttaaacttaacatagaccacctcccctgcgagctaagctggacagccaatgacgggtaagagagtgacatttttcactaacctaagacaggagggccgtcagagctactgcctaatccaaagacgggtaaaagtgataaaaatgtatcactccaacctaagacaggcgcagcttccgagggatttgtcgtctgttttatatatatttaaaagggtgacctgtccggagccgtgctgcccggatgatgtcttggcctctgtttgctctagctctacgcttaagattcaagatggcgaacttcctggttcttctctgtgttgctttcccgccggcgcgaatgtttcccgctcttaggcttacgtggctttcccagttctgcagttgagcatgcgcccagtacttctcccctcccacttactgcctgtgtatataagacaacgcattgccaccattaaacgagacttgatcagaacactgtcttgtctccatttcttgtgtctcttgtcccatccaattcccactccctcctccaggtttcctactgttggtcccgcgggacgggacatt

SEQ ID NO: 42 - protein, 258 aa, Artificial Sequence
  SNV.RBD
MDCLTNLRSAEGKVDQASKILILLVAWWGFGTTAEGYPLQQLWELPCDCSGGYVSSIPTYYTYSLDCGGSTAYLTYGSGTGSWSWGGGFKQQWECVFKPKIIPSVQGQPGPCPSECLQIATQMHSTCYEKTQECTLLGKTYFTAILQKTKLGSYEDGPNKLIQASCTGTVGKPVCWDPVAPVYVSDGGGPTDMIREESVRERLEEIIRHSYPSVQYHPLALPRSRGVDLDPQTSDILEATHQVLNATNPQLAENCWLC

SEQ ID NO: 43 - protein, 567 aa, Artificial Sequence
  SNV.RBD
MDCLTNLRSAEGKVDQASKILILLVAWWGFGTTAEGYPLQQLWELPCDCSGGYVSSIPTYYTYSLDCGGSTAYLTYGSGTGSWSWGGGFKQQWECVFKPKIIPSVQGQPGPCPSECLQIATQMHSTCYEKTQECTLLGKTYFTAILQKTKLGSYEDGPNKLIQASCTGTVGKPVCWDPVAPVYVSDGGGPTDMIREESVRERLEEIIRHSYPSVQYHPLALPRSRGVDLDPQTSDILEATHQVLNATNPKLAENCWLCMTLGTPIPAAIPTNGNVTLDGNCSLSLPFGCNPPGSIDVSCYAGEADNRTGIPVGYVHFTNCTSIQEVTNETSQMGNLTRLCPPPGHVFVCGNNMAYTALPNKWIGLCILASIVPDISIISGEEPIPLPSIEYTARRHKRAVQFIPLLVGLGISGATLAGGTGLGVSVHTYHKLSNQLIEDVQALSGTINDLQDQIDSLAEVVLQNRRGLDLLTAEQGGICLALQEKCCFYANKSGIVRDKIRKLQEDLIERKRALYDNPLWSGLNGFLPYLLPLLGPLFGLILFLTLGPCIMKTLTRIIHDKIQAVKS

SEQ ID NO: 44 - protein, 250 aa, Artificial Sequence
  MPMV.RBD
MNFNYHFIWSLVILSQISQVQAGFGDPREALAEIQQKHGKPCDCAGGYVSSPPINSLTTVSCSTHTAYSVTNSLKWQCVSTPTTPSNTHIGSCPGECNTISYDSVHASCYNHYQQCNIGNKTYLTATITGDRTPAIGDGNVPTVLGTSHNLITAGCPNGKKGQVVCWNSRPSVHISDGGGPQDKARDIIVNKKFEELHRSLFPELSYHPLALPEARGKEKIDAHTLDLLATVHSLLNASQPSLAEDCWLC

SEQ ID NO: 45 - DNA, 8557 bp, Artificial Sequence
  MPMV.RBD
gccaccattaaatgagacttgatcagaacactgtcttgtctccatttcttgtgtctcttgttcccttcaattcccactccctcctccaggttcctactgttgatcccgcgggtcgggacagttggcgcccaacgtggggctggatacgagggaatttcgtgaggaagacgacgcgttcgccggccggcgattaaaagtgaaagtaaactctcttggccgccgcgggaacctgccgcgttggacctgaaagtaagtgttgcgctcggatatggggcaagaattaagccagcatgaacgttatgtagaacaattgaagcaggctttaaagacacggggagtaaaggttaaatatgctgatcttttgaaattttttgattttgtgaaggatacttgtccttggtttccgcaagagggaaccatagatattaaacggtggcgtagagtaggcgactgtttccaagactattacaatacttttggcccggagaaagtcccagtaactgcattctcttactggaacttaattaaagaattgatagataagaaagaagttaacccacaagtaatggctgccgtagcccaaactgaagaaattttaaaaagtaattctcaaacagacctcacaaagacctctcaaaacccagacttggaccttatttcccttgatagcgacgatgaaggagctaaaagttcctctctacaagataaaggtttatcaagtactaaaaaaccaaaaagattcccagttctgttaacagcacaaactagtaaagaccctgaagaccccaacccctcagaggtagactgggacggcttggaagatgaggcagcgaaatatcataatcccgattggcctcccttcctaacccgtccacctccttacaataaagctactccttccgcacccactgtaatggcggttgttaatccaaaagaggagctcaaagaaaaaattgctcaattagaggaacagattaaattagaagagttacaccaggcactaatttccaaattacaaaaactaaaaacagggaatgaaactgtaactcacccagacacagcaggaggcctttctcgcacgcctcactggccagggcaacatatccctaaaggaaaatgttgcgccagtcgagaaaaggaagaacaaatcccaaaagatattttcccagtgactgaaaccgttgatgggcaaggtcaagcctggagacaccataatggttttgattttgccgtcataaaagaattaaaaacagctgcttcccaatatggggctactgccccatacacattagccatagtggaatctgtagcggacaattggcttacccctacagattggaatacgcttgttagggcagtcctctcaggaggagatcacttactgtggaaatctgagttttttgaaaattgcagagatacggctaaaagaaaccaacaagccggtaatggctgggattttgacatgttaacaggttcgggtaattattccagcaccgatgcacaaatgcagtatgatccaggattgtttgctcaaattcaagcggctgctacaaaagcctggagaaaacttcccgttaagggagacccaggagcctcccttacaggagtcaaacaaggacccgatgagccatttgcagatttcgtacacagacttataacaactgctgggagaatctttggaagtgctgaggccggtgtagactatgtaaaacaactagcatatgaaaatgctaatccagcttgtcaggcagccattcgcccctatagaaagaagacagatttaactggctatatccgtctttgctcggatattgggccctcttatcagcaaggcctggccatggccgccgcctttagcgggcagactgtaaaagattttcttaacaacaaaaataaagagaaaggagggtgttgctttaaatgcggtaaaaaaggacactttgcaaaaaattgtcatgaacatgcacataacaatgctgaaccaaaagttcccggactctgccctagatgtaaaagagggaaacattgggccaatgaatgcaaatccaaaactgataatcaaggaaacccaataccaccccatcagggaaacgggtggaggggccagccccaggccccgaaacaagcttatggggcagtcagctttgttccagccaacaaaaacaacccatttcaaagcttaccagagccaccccaggaagtgcaggattggacctctgttccacctcccacacagtattaacgcctgaaatggggccccaagcgttaagcactggaatatatggaccactgcctcccaacacttttggattaatcctaggccgaagtagcattactatgaagggtctacaagtttatccaggagtaattgataatgactataccggagaaattaaaattatggcaaaagctgttaacaatattgttactgtctctcaaggcaacagaatagctcaattaatcctcctgcctctgatcgagacagacaataaggtacaacaaccttatagaggacaaggaagttttggatcctcagacatatattgggtccaacctattacttgtcaaaaaccttccttaacattatggttagatgacaaaatgttcacaggcttaatagatacgggggctgatgtcacaattatcaagctggaggactggcctcctaattggcctataacagataccttaaccaatttaagaggaataggacaaagtaacaaccctaaacaaagttctaaatatcttacttggagagataaagaaaacaattctggtctcatcaaaccgtttgttattcctaacttacctgtcaatctttggggccgagatttactttctcaaatgaaaattatgatgtgtagccccaatgacatagtaactgctcaaatgttagcccagggctacagcccaggaaaagggttaggaaaaaaggaaaatggcattctacatcctatcccaaatcaaggacaatctaacaaaaaaggttttggaaatttttaactgcggccattgacatacttgcaccccaacagtgcgctgaacccatcacgtggaaatcagacgaacctgtctgggttgatcagtggccattaaccaatgacaaacttgctgctgcccaacagttagtgcaagaacagttagaggcaggacatattactgaaagtagttctccctggaacactcccatatttgttataaaaaagaaatctggtaaatggaggctcttacaagatttacgagccgttaatgccactatggtattaatgggagctttacaacctggattaccctccccggtggctatcccacaagggtatcttaaaataattattgatctcaaggattgtttcttttctattccccttcatcctagtgaccaaaaaagatttgccttcagcctaccatccacaaattttaaagaacctatgcaacgttttcagtggaaggttttaccacaaggtatggccaacagtcctaccttatgtcaaaaatatgtggccacagccatacataaggttagacatgcctggaaacaaatgtatattatacattacatggatgacatcctaatagctggtaaagatggacaacaagttttgcaatgctttgatcaactcaaacaagagttgactgcagctgggttacatatagccccagaaaaagttcaattacaagatccctacacatatttaggatttgaacttaatggtcctaaaatcactaatcaaaaagcagtcattcgtaaagataaattacagactcttaatgatttccaaaaacttttaggagacatcaattggctcagaccatatctaaaactcactactggagacttaaaacccttattcgacacccttaaaggagactctgaccccaattcccatagatccttatcaaaagaagctcttgcctcacttgaaaaggtagagacagccattgcagaacaattcgttactcacataaattattcactaccattaattttcctcatattcaacacagccctgacacctactggtttgttttggcaagacaatcctattatgtggatccacctgcctgcatcccctaaaaaggtgttacttccctactacgacgctatagcagatttaatcatactagggagagaccatagtaaaaaatattttggaattgaaccctctacaatcatacaaccatattctaagtctcagattgattggttaatgcaaaacactgaaatgtggccaattgcctgtgcctcctttgttggcatcctagataaccattatccaccaaataaacttatccagttctgtaaactacatacctttgttttccctcaaatcattagtaaaacacccttaaacaatgccttattagtttttactgatggctcttccactgggatggccgcatatactcttactgataccaccatcaaattccaaactaatcttaattcggctcaactagtagaactacaagctttaattgcagtcttatcagccttccctaatcaacctcttaatatttacactgacagtgcttacttagcccactcaatacccctacttgaaactgtcgcacaaattaaacacatatcagaaacagctaaactgttcctacagtgccagcaactcatatacaatagatccatacctttttatattggacatgtcagggcccattctggactacctggacccatagctcaaggcaaccaacgagctgacttggcaactaaaatcgtggctagtaacataaacacaaacctcgaatcagctcaaaatgctcataccttacatcacctcaatgcccagactttaagacttatgtttaacattcctagagaacaagctagacaaattgttaagcaatgtcctatatgtgtaacttatctaccagtccctcatttaggagttaatcctaggggattatttcccaacatgatttggcaaatggatgttacacactactcagaatttggcaatttaaaatatattcatgtatctatagatacattcagtggattcctactggccactctacaaacaggagaaactacaaaacatgtcataacccatttactccattgcttctctattattggactccctaaacaaattaaaacggataacggtcctggatacacctctaaaaattttcaagaattttgctccacacttcaaattaaacatattactggaatcccctataacccccaaggccaaggaatagttgaaagagcccacttatctcttaaaaccaccattgaaaagataaaaaagggggaatggtaccctaggaagggtacccccaggaacatcctcaatcatgcactctttattctaaattttttaaatttagatgatcaaaataaatcagcagctgatcgtttttggcataataaccccaaaaaacaatttgccatggtaaaatggaaagatccattagataatacatggcatggccccgatccagtgttaatttggggcagaggttcagtctgtgtttactctcaaacctatgatgccgctagatggctaccagaacggttagtaagacaggtgtctaacaataaccaatccagggagtgattctctccctgagatcgctctttcccttgttcacagatatgaacttcaattatcatttcatctggagcttagtgatactatctcaaatatctcaagttcaagccggttttggagatccgcgtgaagccctggcagaaatacaacaaaaacatggtaaaccttgtgactgtgctggaggatatgtttcctccccaccgattaactctcttacaactgtttcttgctctactcatactgcttattcagtgacaaactccctaaaatggcagtgtgtgtcaactcccactacccctagcaatacacatataggaagttgtcccggtgaatgcaacacgatctcatatgattctgtacatgcctcttgctataaccactatcaacaatgtaacattggtaataaaacatatctcactgccactataactggagatagaactcctgccattggtgacgggaatgtccctacagtactagggactagtcacaacctcattacagcaggctgtcccaatggtaaaaagggccaagtggtctgttggaatagccgaccttctgttcatatatctgatggaggagggcctcaagataaggcccgcgacattatagtaaataaaaagtttgaggaattgcacaggtcgctgttcccagaactttcttaccatcctctggccttgcccgaagcccgtggtaaagaaaaaattgacgcacacactcttgatctccttgccactgtacatagtttactcaatgcttcccaacccagtttagccgaagattgctggctgtgcttacagtcaggagatcccgttcctcttgccctgccctataatgatacactctgctctaactttgcctgtttatctaatcactcctgccctttaacccccccttttttagtacagccctttaacttcactgattccaattgcctttacgctcattatcaaaacaactcatttgacatagatgtaggtctagctagctttactaattgctctagctattataacgtttctacagcctccaaaccctctaattccctatgcgccccaaacagctcggtttttgtatgcggtaacaataaggcatacacttatctacccacaaattggacgggaagttgtgtacttgctactcttttgcccgatatagacatcattccaggtagtgagcctgtccccattccagctattgatcattttttaggcaaagccaaaagagcaatccaacttatccccctgttcgtagggttaggtataactactgcagtatctactggggctgctggtctaggggtttccatcactcaatatacaaaattatctcatcaactaatatcagatgttcaagctatttctagcactatacaagatctccaagatcaggtagactctctagcagaagtagtactgcaaaacagaagaggattagatctacttacagcagagcagggaggtatctgcttagccttacaggaaaaatgttgtttctacgccaataaatctggaatcgtcagagacaagattaaaaacctacaagacgacttagaaagacgccgaagacaactgatcgacaacccattttggaccagttttcatggattcctcccttatgttatgcccctattaggccctttgctttgcttattgcttgtgttatctttcggtccaattattttcaacaagcttatgacctttattaaacatcaaattgagagcatccaggccaaacctatacaagtccattatcatcgccttgaacaagaagacagtggtggctcatatttgaccttaacataggccacctcccctgtgagctagactggacagccaatgacgggtaagagagtgacatttctcactaacctaagacaggagggccgtcaaagctactgcctaatccaatgacgggtaatagtgacaagaaatgtatcactccaacctaagacaggcgcagcctccgagggatgtgtcttttgttttttataattaaaaagggtgacatgtccggagccgtgctgcccggatgatgtcttggcctctgtttgctctagctccatgttatgaatttaagatggcgtatttcctggttcttctccgtcttactttcccgccggcgcgaatgtttcccgctcttgggcttacgtggctttccttgctctgctactgagcatgcgcccagtatctttcccctcccacttgctgcctgtgtatataaggcaacacattgccaccattaaatgagacttgatcagaacactgtcttgtctccatttcttgtgtctcttgttcccttcaattcccactccctcctccaggttcctactgttgatcccgcgggtcgggacagttttcgttttctgtccggagccgtgctgcccggatgatgtcttggcctctgtttgctctagctccatgttatgaatttaagatggcgtatttcctggttcttctccgtcttactttcccgccggcgcgaatgtttcccgctcttgggcttacgtggctttccttgctctgctactgagcatgcgcccagtatctttcccctcccacttgctgcctgtgtatataaggcaacacattgccaccattaaatgagacttgatcagaacactgtcttgtctccatttcttgtgtctcttgttcccttcaattcccactccctcctccaggttcctactgttgatcccgcgggtcgggacagttggcgcccaacgtggggcacgaacccacgaccctgggattaagagtcccatgctctaccgactggatgatgtcttggcctctgtttgctctagctccatgttatgaatttaagatggcgtatttcctggttcttctccgtcttactttcccgccggcgcgaatgtttcccgctcttgggcttacgtggctttccttgctctgctactgagcatgcgcccagtatctttcccctcccacttgctgcctgtgtatataaggcaacacatt

SEQ ID NO: 46 - protein, 189 aa, Artificial Sequence
  HERV-W.RBD
MALPYHIFLFTVLLPSFTLTAPPPCRCMTSSSPYQEFLWRMQRPGNIDAPSYRSLCKGTPTFTAHTHMPRNCYHSATLCMHANTHYWTGKMINPSCPGGLGVTVCWTYFTQTGMSDGGGVQDQAREKHVKEVISQLTRVHGTSSPYKGLDLSKLHETLRTHTRLVSLFNTTLTGLHEVSAQNPTNCWIC

SEQ ID NO: 47 - protein, 293 aa, Artificial Sequence
  Xeno.RBD
MEGSAFSKPLKDKINPWGPLIVMGILVRAGASVQRDSPHQIFNVTWRVTNLMTGQTANATSLLGTMTDTFPKLYFDLCDLVGDYWDDPEPDIGDGCRTPGGRRRTRLYDFYVCPGHTVPIGCGGPGEGYCGKWGCETTGQAYWKPSSSWDLISLKRGNTPKDQGPCYDSSVSSGVQGATPGGRCNPLVLEFTDAGRKASWDAPKVWGLRLYRSTGADPVTRFSLTRQVLNVGPRVPIGPNPVITDQLPPSQPVQIMLPRPPHPPPSGTVSMVPGAPPPSQQPGTGDRLLNLVE

SEQ ID NO: 48 - protein, 238 aa, Artificial Sequence
  Xeno.RBD
MEGSAFSKPLKDKINPWGPLIVMGILVRAGASVQRDSPHQIFNVTWRVTNLMTGQTANATSLLGTMTDTFPKLYFDLCDLVGDYWDDPEPDIGDGCRTPGGRRRTRLYDFYVCPGHTVPIGCGGPGEGYCGKWGCETTGQAYWKPSSSWDLISLKRGNTPKDQGPCYDSSVSSGVQGATPGGRCNPLVLEFTDAGRKASWDAPKVWGLRLYRSTGADPVTRFSLTRQVLNVGPRVPIG

SEQ ID NO: 49 - protein, 223 aa, Artificial Sequence
  RD114.RBD
MKLPAGMVILCSLIIVRAGFDDPRKAIALVQKQHGKPCECSGGQVSEAPPNSIQQVTCPGKTAYLMTNQKWKCRVTPKNLTPSGGELQNCPCNTFQDSMHSSCYTEYRQCRANNKTYYTATLLKIRSGSLNEVQILQNPNQLLQSPCRGSINQPVCWSATAPIHISDGGGPLDTKRVWTVQKRLEQIHKAMHPELQYHPLALPKVRDDLSLDARTFDILNTTF

SEQ ID NO: 50 - DNA, 993 bp, Artificial Sequence
  RD114.RBD
atgaaacccccagcgggaatggtctttctgtgggtcctcacaagcttgggggcgggaattggagctaaaattgtcaaagaggggaacccacatcaggtttataccttgacttggcaaatctactcccagagcggggaagttgtctgggaggtccaaggtaaccatgcgcttaatacttggtggcccccacttacccctgatttttgccagctggcagctggattagacacttgggatatcccagctagaagccccaagaacctgcagtcctacatgggggaaagaatccagcagatgactgcccatggatgcagtagtcccactgccagatgtagattagcccaggcagagttctatgtctgtcctcgagacaatagggatagggccactgcccaccgatgtgggggatatgaagaatatttctgctcggcatggggctgcgaaactactggcgatgcctactggcaacctacctcttcctgggacttaatcaccattacaagaggttacaccaaacctgaccccgatggacacacttgctactataaaaagggcacagaagggtatcatcattggataagtcccctgtctctacctcttaagattacctttacagattcaggaaaacgggctctcggatggcagacgggctatacatggggactccgatggtacctaccgggaaaagatagggggattgttctaaaaatcaaattaaaaatagatacaatcacccaaaccgtaggtcccaacctagtattggccgatcaaaaagctccggtccagctagccatcccagtccagccaccaagggccccaactcagacaccgggaattaaccctgttaattccactctaagccccagtctaggatacccgaccccccctctcgaccgggcacaaggagataggctcctaaaccttgtacaaggggtatacttaactctcaaccttacggccccaaatcaaactcaggactgttggctctgccta

SEQ ID NO: 51 - protein, 352 aa, Artificial Sequence
  HERV-W.RBD fused to a mouse Fc fragment
MALPYHIFLFTVLLPSFTLTAPPPCRCMTSSSPYQEFLWRMQRPGNIDAPSYRSLSKGTPTFTAHTHMPRNCYHSATLCMHANTHYWTGKMINPSCPGGLGVTVCWTYFTQTGMSDGGGVQGSVDVPRDCGCKPCICTVPEVSSVFIFPPKPKDVLTITLTPKVTCVVVDISKDDPEVQFSWFVDDVEVHTAQTQPREEQFNSTFRSVSELPIMHQDWLNGKEFKCRVNSAAFPAPIEKTISKTKGRPKAPQVYTIPPPKEQMAKDKVSLTCMITDFFPEDITVEWQWNGQPAENYKNTQPIMDTDGSYFVYSKLNVQKSNWEAGNTFTCSVLHEGLHNHHTEKSLSHSPGK

SEQ ID NO: 52 - protein, 470 aa, Artificial Sequence
  Xeno.RBD fused to a rabbit Fc fragment
MLVMEGSAFSKPLKDKINPWGPLIVMGILVRAGASVQRDSPHQIFNVTWRVTNLMTGQTANATSLLGTMTDTFPKLYFDLCDLVGDYWDDPEPDIGDGCRTPGGRRRTRLYDFYVCPGHTVPIGCGGPGEGYCGKWGCETTGQAYWKPSSSWDLISLKRGNTPKDQGPCYDSSVSSGVQGATPGGRCNPLVLEFTDAGRKASWDAPKVWGLRLYRSTGADPVTRFSLTRQVLNVGPRVPIGSAPSTCSKPTCPPPELLGGPSVFIFPPKPKDTLMISRTPEVTCVVVDVSQDDPEVQFTWYINNEQVRTARPPLREQQFNSTIRVVSTLPITHQDWLRGKEFKCKVHNKALPAPIEKTISKARGQPLEPKVYTMGPPREELSSRSVSLTCMINGFYPSDISVEWEKNGKAEDNYKTTPAVLDSDGSYFLYNKLSVPTSEWQRGDVFTCSVMHEALHNHYTQKSISRSPGK

SEQ ID NO: 53 - protein, 523 aa, Artificial Sequence
  Xeno.RBD fused to a rabbit Fc fragment
MEGSAFSKPLKDKINPWGPLIVMGILVRAGASVQRDSPHQIFNVTWRVTNLMTGQTANATSLLGTMTDTFPKLYFDLCDLVGDYWDDPEPDIGDGCRTPGGRRRTRLYDFYVCPGHTVPIGCGGPGEGYCGKWGCETTGQAYWKPSSSWDLISLKRGNTPKDQGPCYDSSVSSGVQGATPGGRCNPLVLEFTDAGRKASWDAPKVWGLRLYRSTGADPVTRFSLTRQVLNVGPRVPIGPNPVITDQLPPSQPVQIMLPRPPHPPPSGTVSMVPGAPPPSQQPGTGDRLLNLVEGSAPSTCSKPTCPPPELLGGPSVFIFPPKPKDTLMISRTPEVTCVVVDVSQDDPEVQFTWYINNEQVRTARPPLREQQFDCTIRVVSTLPIAHQDWLRGKEFKCKVHNKALPAPIEKTISKARGQPLEPKVYTMGPPREELSSRSVSLTCMINGFYPSDISVEWEKNGKAEDNYKTTPAVLDSDGSYFLYSKLSVPTSEWQRGDVFTCSVMHEALHNHYTQKSISRSPGK

SEQ ID NO: 54 - protein, 453 aa, Artificial Sequence
  RD114.RBD fused to a mouse Fc fragment
MKLPTGMVILCSLIIVRAGFDDPRKAIALVQKQHGKPCECSGGQVSEAPPNSIQQVTCPGKTAYLMTNQKWKCRVTPKISPSGGELQNCPCNTFQDSMHSSCYTEYRQCRRINKTYYTATLLKIRSGSLNEVQILQNPNQLLQSPCRGSINQPVCWSATAPIHISDGGGPLDTKRVWTVQKRLEQIHKAMTPELQYHPLALPKVRDDLSLDARTFDILNTTFGSVDVPRDCGCKPCICTVPEVSSVFIFPPKPKDVLTITLTPKVTCVVVDISKDDPEVQFSWFVDDVEVHTAQTQPREEQFNSTFRSVSELPIMHQDWLNGKEFKCRVNSAAFPAPIEKTISKTKGRPKAPQVYTIPPPKEQMAKDKVSLTCMITDFFPEDITVEWQWNGQPAENYKNTQPIMDTDGSYFVYSKLNVQKSNWEAGNTFTCSVLHEGLHNHHTEKSLSHSPGK

SEQ ID NO: 55 - protein, 454 aa, Artificial Sequence
  RD114.RBD fused to a mouse Fc fragment
MKLPAGMVILCSLIIVRAGFDDPRKAIALVQKQHGKPCECSGGQVSEAPPNSIQQVTCPGKTAYLMTNQKWKCRVTPKNLTPSGGELQNCPCNTFQDSMHSSCYTEYRQCRANNKTYYTATLLKIRSGSLNEVQILQNPNQLLQSPCRGSINQPVCWSATAPIHISDGGGPLDTKRVWTVQKRLEQIHKAMHPELQYHPLALPKVRDDLSLDARTFDILNTTFGSVDVPRDCGCKPCICTVPEVSSVFIFPPKPKDVLTITLTPKVTCVVVDISKDDPEVQFSWFVDDVEVHTAQTQPREEQFNSTFRSVSELPIMHQDWLNGKEFKCRVNSAAFPAPIEKTISKTKGRPKAPQVYTIPPPKEQMAKDKVSLTCMITDFFPEDITVEWQWNGQPAENYKNTQPIMDTDGSYFVYSKLNVQKSNWEAGNTFTCSVLHEGLHNHHTEKSLSHSPGK